European Patent Application EP 4 183 796 A1, published May 24, 2023. Title: Thermostable FGF10 polypeptide or fragment thereof and use thereof. Applicant: Enantis s.r.o. The sequence listing filed with the application follows.

SEQUENCE LISTING (18 sequences)

SEQ ID NO: 1 - protein, 208 aa, Artificial Sequence
  Human FGF10
MWKWILTHCASAFPHLPGCCCCCFLLLFLVSSVPVTCQALGQDMVSPEATNSSSSSFSSPSSAGRHVRSYNHLQGDVRWRKLFSFTKYFLKIEKNGKVSGTKKENCPYSILEITSVEIGVVAVKAINSNYYLAMNKKGKLYGSKEFNNDCKLKERIEENGYNTYASFNWQHNGRQMYVALNGKGAPRRGQKTRRKNTSAHFLPMVVHS

SEQ ID NO: 2 - protein, 37 aa, Artificial Sequence
  N-terminal signal peptide of human FGF10
MWKWILTHCASAFPHLPGCCCCCFLLLFLVSSVPVTC

SEQ ID NO: 3 - protein, 140 aa, Artificial Sequence
  Ser69-Ser208 fragment of SEQ ID NO: 1 + L152F
SYNHLQGDVRWRKLFSFTKYFLKIEKNGKVSGTKKENCPYSILEITSVEIGVVAVKAINSNYYLAMNKKGKLYGSKEFNNDCKFKERIEENGYNTYASFNWQHNGRQMYVALNGKGAPRRGQKTRRKNTSAHFLPMVVHS

SEQ ID NO: 4 - protein, 68 aa, Artificial Sequence
  N-terminal Met1-Arg68 part of SEQ ID NO: 1
MWKWILTHCASAFPHLPGCCCCCFLLLFLVSSVPVTCQALGQDMVSPEATNSSSSSFSSPSSAGRHVR

SEQ ID NO: 5 - protein, 169 aa, Artificial Sequence
  Leu40-Ser208 fragment of SEQ ID NO: 1+L152F
LGQDMVSPEATNSSSSSFSSPSSAGRHVRSYNHLQGDVRWRKLFSFTKYFLKIEKNGKVSGTKKENCPYSILEITSVEIGVVAVKAINSNYYLAMNKKGKLYGSKEFNNDCKFKERIEENGYNTYASFNWQHNGRQMYVALNGKGAPRRGQKTRRKNTSAHFLPMVVHS

SEQ ID NO: 6 - protein, 39 aa, Artificial Sequence
  N-terminal Met1-Ala39 part of SEQ ID NO: 1
MWKWILTHCASAFPHLPGCCCCCFLLLFLVSSVPVTCQA

SEQ ID NO: 7 - protein, 169 aa, Artificial Sequence
  Leu40-Ser208 fragment of SEQ ID NO: 1 + L152F+V123I
LGQDMVSPEATNSSSSSFSSPSSAGRHVRSYNHLQGDVRWRKLFSFTKYFLKIEKNGKVSGTKKENCPYSILEITSVEIGVVAIKAINSNYYLAMNKKGKLYGSKEFNNDCKFKERIEENGYNTYASFNWQHNGRQMYVALNGKGAPRRGQKTRRKNTSAHFLPMVVHS

SEQ ID NO: 8 - protein, 169 aa, Artificial Sequence
  Leu40-Ser208 fragment of SEQ ID NO: 1 + L152F+Q175E
LGQDMVSPEATNSSSSSFSSPSSAGRHVRSYNHLQGDVRWRKLFSFTKYFLKIEKNGKVSGTKKENCPYSILEITSVEIGVVAVKAINSNYYLAMNKKGKLYGSKEFNNDCKFKERIEENGYNTYASFNWQHNGREMYVALNGKGAPRRGQKTRRKNTSAHFLPMVVHS

SEQ ID NO: 9 - protein, 169 aa, Artificial Sequence
  Leu40-Ser208 fragment of SEQ ID NO: 1 + L152F+N181D
LGQDMVSPEATNSSSSSFSSPSSAGRHVRSYNHLQGDVRWRKLFSFTKYFLKIEKNGKVSGTKKENCPYSILEITSVEIGVVAVKAINSNYYLAMNKKGKLYGSKEFNNDCKFKERIEENGYNTYASFNWQHNGRQMYVALDGKGAPRRGQKTRRKNTSAHFLPMVVHS

SEQ ID NO: 10 - protein, 169 aa, Artificial Sequence
  Leu40-Ser208 fragment of SEQ ID NO: 1 + L152F+V123I+Q175E
LGQDMVSPEATNSSSSSFSSPSSAGRHVRSYNHLQGDVRWRKLFSFTKYFLKIEKNGKVSGTKKENCPYSILEITSVEIGVVAIKAINSNYYLAMNKKGKLYGSKEFNNDCKFKERIEENGYNTYASFNWQHNGREMYVALNGKGAPRRGQKTRRKNTSAHFLPMVVHS

SEQ ID NO: 11 - protein, 169 aa, Artificial Sequence
  Leu40-Ser208 fragment of SEQ ID NO: 1 + L152F+V123I+N181D
LGQDMVSPEATNSSSSSFSSPSSAGRHVRSYNHLQGDVRWRKLFSFTKYFLKIEKNGKVSGTKKENCPYSILEITSVEIGVVAIKAINSNYYLAMNKKGKLYGSKEFNNDCKFKERIEENGYNTYASFNWQHNGRQMYVALDGKGAPRRGQKTRRKNTSAHFLPMVVHS

SEQ ID NO: 12 - protein, 169 aa, Artificial Sequence
  Leu40-Ser208 fragment of SEQ ID NO: 1 + L152F+Q175E+N181D
LGQDMVSPEATNSSSSSFSSPSSAGRHVRSYNHLQGDVRWRKLFSFTKYFLKIEKNGKVSGTKKENCPYSILEITSVEIGVVAVKAINSNYYLAMNKKGKLYGSKEFNNDCKFKERIEENGYNTYASFNWQHNGREMYVALDGKGAPRRGQKTRRKNTSAHFLPMVVHS

SEQ ID NO: 13 - protein, 169 aa, Artificial Sequence
  FGF10-STAB
LGQDMVSPEATNSSSSSFSSPSSAGRHVRSYNHLQGDVRWRKLFSFTKYFLKIEKNGKVSGTKKENCPYSILEITSVEIGVVAIKAINSNYYLAMNKKGKLYGSKEFNNDCKFKERIEENGYNTYASFNWQHNGREMYVALDGKGAPRRGQKTRRKNTSAHFLPMVVHS

SEQ ID NO: 14 - protein, 169 aa, Artificial Sequence
  Leu40-Ser208 fragment of SEQ ID NO: 1, FGF10-wt
LGQDMVSPEATNSSSSSFSSPSSAGRHVRSYNHLQGDVRWRKLFSFTKYFLKIEKNGKVSGTKKENCPYSILEITSVEIGVVAVKAINSNYYLAMNKKGKLYGSKEFNNDCKLKERIEENGYNTYASFNWQHNGRQMYVALNGKGAPRRGQKTRRKNTSAHFLPMVVHS

SEQ ID NO: 15 - protein, 190 aa, Artificial Sequence
  Recombinant human FGF10-wt
MGSSHHHHHHSSGLVPRGSHMLGQDMVSPEATNSSSSSFSSPSSAGRHVRSYNHLQGDVRWRKLFSFTKYFLKIEKNGKVSGTKKENCPYSILEITSVEIGVVAVKAINSNYYLAMNKKGKLYGSKEFNNDCKLKERIEENGYNTYASFNWQHNGRQMYVALNGKGAPRRGQKTRRKNTSAHFLPMVVHS

SEQ ID NO: 16 - protein, 136 aa, Artificial Sequence
  FGF10 from Falco peregrinus having 88% sequence identity with SEQ ID NO: 3 and SEQ ID NO: 5
LQGDVRKRKLYSYNKYFLKIEKNGKVSGTKKENCPFSILEITSVEIGVVAVKSIKSNYYLAMNKKGKVYGSKEFNSDCKLKERIEENGYNTYASLNWKHNGRQMFVALNGRGATKRGQKTRRKNTSAHFLPMVVMS

SEQ ID NO: 17 - protein, 136 aa, Artificial Sequence
  FGF10-Fp+L152F
LQGDVRKRKLYSYNKYFLKIEKNGKVSGTKKENCPFSILEITSVEIGVVAVKSIKSNYYLAMNKKGKVYGSKEFNSDCKFKERIEENGYNTYASLNWKHNGRQMFVALNGRGATKRGQKTRRKNTSAHFLPMVVMS

SEQ ID NO: 18 - DNA, 584 bp, Artificial Sequence
  Nucleotide sequence of recombinant human FGF10-wt
ccatgggcagcagccatcatcatcatcatcacagcagcggcctggtgccgcgcggcagccatatgctgggtcaagatatggttagtccggaagcaaccaatagcagcagcagctcatttagcagcccgagcagcgcaggtcgtcatgttcgtagctataatcatctgcagggtgatgttcgttggcgtaaactgtttagctttaccaaatacttcctgaaaatcgaaaagaacggtaaagttagcggcaccaaaaaagaaaattgcccgtatagcattctggaaattaccagcgttgaaattggtgttgttgccgtgaaagcaatcaacagcaactattatctggccatgaacaaaaaaggcaaactgtatggtagcaaagagttcaacaacgactgcaaactgaaagaacgcattgaagaaaatggctataatacctatgccagctttaactggcagcataatggtcgtcagatgtatgttgcactgaatggtaaaggtgcaccgcgtcgtggtcagaaaacccgtcgtaaaaataccagcgcacattttctgccgatggttgttcatagctaatagctcgag